European Patent Application EP 4 684 838 A1, published January 28, 2026. Title: USE OF POLYPEPTIDE-IN37 AND SKINCARE PRODUCT CONTAINING POLYPEPTIDE-IN37. Applicant: Ideal Medical Technology Development Co., Ltd. Application EP. The sequence listing filed with the application follows.

SEQUENCE LISTING (1 sequence)

SEQ ID NO: 1 - protein, 13 aa, synthetic construct
  SITE 4: note = D-phenylalanine
  SITE 6: note = D-phenylalanine
  SITE 8: note = D-phenylalanine
  SITE 9: note = D-phenylalanine
  SITE 11: note = D-phenylalanine
  MOD_RES 13: note = AMIDATION
ILPXKXPXXPXRR